European Patent Specification EP 3 741 850 B1, published May 20, 2026. Title: POLIPEPTÍDEO COM ATIVIDADE ASPARAGINASE, CASSETE DE EXPRESSÃO, VETOR DE EXPRESSÃO, CÉLULA HOSPEDEIRA, COMPOSIÇÃO FARMACÊUTICA, MÉTODOS PARA PRODUZIR UM POLIPEPTÍDEO COM ATIVIDADE ASPARAGINASE E PARA PREVENIR OU TRATAR CÂNCER, E, USO DE UM POLIPEPTÍDEO. Applicant: FUNDAÇÃO OSWALDO CRUZ. The sequence listing filed with the application follows.

SEQUENCE LISTING (11 sequences)

SEQ ID NO: 1 - protein, 308 aa, Homo sapiens
MNPIVVVHGGGAGPISKDRKERVHQGMVRAATVGYGILREGGSAVDAVEGAVVALEDDPEFNAGCGSVLNTNGEVEMDASIMDGKDLSAGAVSAVQCIANPIKLARLVMEKTPHCFLTDQGAAQFAAAMGVPEIPGEKLVTERNKKRLEKEKHEKGAQKTDCQKNLGTVGAVALDCKGNVTYATSTGGIVNKMVGRVGDSPCLGAGGYADNDIGAVSTTGHGESILKVNLARLTLFHIEQGKTVEEAADLSLGYMKSRVKGLGGLIVVSKTGDWVAKWTSTSMPWAAAKDGKLHFGIDPDDTTITDLP

SEQ ID NO: 2 - DNA, 1332 bp, Homo sapiens
cggggagcggcggtaccgggcggctgcggggctggctcgacccagcttgaggtctcggcgtccgcgtcctgcggtgccctgggatccgccgacatgaatcccatcgtagtggtccacggcggcggagccggtcccatctccaaggatcggaaggagcgagtgcaccagggcatggtcagagccgccaccgtgggctacggcatcctccgggagggcgggagcgccgtggatgccgtagagggagctgtcgtcgccctggaagacgatcccgagttcaacgcaggttgtgggtctgtcttgaacacaaatggtgaggttgaaatggatgctagtatcatggatggaaaagacctgtctgcaggagcagtgtccgcagtccagtgtatagcaaatcccattaaacttgctcggcttgtcatggaaaagacacctcattgctttctgactgaccaaggcgcagcgcagtttgcagcagctatgggggttccagagattcctggagaaaaactggtgacagagagaaacaaaaagcgcctggaaaaagagaagcatgaaaaaggtgctcagaaaacagattgtcaaaaaaacttgggaaccgtgggtgctgttgccttggactgcaaagggaatgtaacctacgcaacctccacaggcggtatcgttaataaaatggtcggccgcgttggggactcaccgtgtctaggagctggaggttatgccgacaatgacatcggagccgtctcaaccacagggcatggggaaagcatcctgaaggtgaacctggctagactcaccctgttccacatagaacaaggaaagacggtagaagaggctgcggacctatcgttgggttatatgaagtcaagggttaaaggtttaggtggcctcatcgtggttagcaaaacaggagactgggtggcaaagtggacctccacctccatgccctgggcagccgccaaggacggcaagctgcactttggaattgatcctgacgatactactatcaccgaccttccctaagccgctggaagattgtattccagatgctagcttagaggtcaagtacagtctcctcatgagacatagcctaatcaattagatctagaattggaaaaattgtcccgtctgtcacttgttttgttgccttaataagcatctgaatgtttggttgtggggcgggttttgaagcgatgagagaaatgcccgtattaggaggattacttgagccctggaggtcaaagctgaggtgagccatgattactccactgcactccagcctgggcaacagagccaggccctgtatcaaaaaaaaaaaaaaaaaaaaaaaaaaaa

SEQ ID NO: 3 - protein, 308 aa, Sequência Artificial
  Substituição de G por E na posição 10 da sequência selvagem
MNPIVVVHGEGAGPISKDRKERVHQGMVRAATVGYGILREGGSAVDAVEGAVVALEDDPEFNAGCGSVLNTNGEVEMDASIMDGKDLSAGAVSAVQCIANPIKLARLVMEKTPHCFLTDQGAAQFAAAMGVPEIPGEKLVTERNKKRLEKEKHEKGAQKTDCQKNLGTVGAVALDCKGNVTYATSTGGIVNKMVGRVGDSPCLGAGGYADNDIGAVSTTGHGESILKVNLARLTLFHIEQGKTVEEAADLSLGYMKSRVKGLGGLIVVSKTGDWVAKWTSTSMPWAAAKDGKLHFGIDPDDTTITDLP

SEQ ID NO: 4 - protein, 308 aa, Sequência Artificial
  Substituição de G por D na posição 10 da sequência selvagem
MNPIVVVHGDGAGPISKDRKERVHQGMVRAATVGYGILREGGSAVDAVEGAVVALEDDPEFNAGCGSVLNTNGEVEMDASIMDGKDLSAGAVSAVQCIANPIKLARLVMEKTPHCFLTDQGAAQFAAAMGVPEIPGEKLVTERNKKRLEKEKHEKGAQKTDCQKNLGTVGAVALDCKGNVTYATSTGGIVNKMVGRVGDSPCLGAGGYADNDIGAVSTTGHGESILKVNLARLTLFHIEQGKTVEEAADLSLGYMKSRVKGLGGLIVVSKTGDWVAKWTSTSMPWAAAKDGKLHFGIDPDDTTITDLP

SEQ ID NO: 5 - protein, 308 aa, Sequência Artificial
  Substituição de G por H na posição 10 da sequência selvagem
MNPIVVVHGHGAGPISKDRKERVHQGMVRAATVGYGILREGGSAVDAVEGAVVALEDDPEFNAGCGSVLNTNGEVEMDASIMDGKDLSAGAVSAVQCIANPIKLARLVMEKTPHCFLTDQGAAQFAAAMGVPEIPGEKLVTERNKKRLEKEKHEKGAQKTDCQKNLGTVGAVALDCKGNVTYATSTGGIVNKMVGRVGDSPCLGAGGYADNDIGAVSTTGHGESILKVNLARLTLFHIEQGKTVEEAADLSLGYMKSRVKGLGGLIVVSKTGDWVAKWTSTSMPWAAAKDGKLHFGIDPDDTTITDLP

SEQ ID NO: 6 - DNA, 1332 bp, Sequência Artificial
  Substituição de g por a na posição 29 da sequência selvagem
cggggagcggcggtaccgggcggctgcgaggctggctcgacccagcttgaggtctcggcgtccgcgtcctgcggtgccctgggatccgccgacatgaatcccatcgtagtggtccacggcggcggagccggtcccatctccaaggatcggaaggagcgagtgcaccagggcatggtcagagccgccaccgtgggctacggcatcctccgggagggcgggagcgccgtggatgccgtagagggagctgtcgtcgccctggaagacgatcccgagttcaacgcaggttgtgggtctgtcttgaacacaaatggtgaggttgaaatggatgctagtatcatggatggaaaagacctgtctgcaggagcagtgtccgcagtccagtgtatagcaaatcccattaaacttgctcggcttgtcatggaaaagacacctcattgctttctgactgaccaaggcgcagcgcagtttgcagcagctatgggggttccagagattcctggagaaaaactggtgacagagagaaacaaaaagcgcctggaaaaagagaagcatgaaaaaggtgctcagaaaacagattgtcaaaaaaacttgggaaccgtgggtgctgttgccttggactgcaaagggaatgtaacctacgcaacctccacaggcggtatcgttaataaaatggtcggccgcgttggggactcaccgtgtctaggagctggaggttatgccgacaatgacatcggagccgtctcaaccacagggcatggggaaagcatcctgaaggtgaacctggctagactcaccctgttccacatagaacaaggaaagacggtagaagaggctgcggacctatcgttgggttatatgaagtcaagggttaaaggtttaggtggcctcatcgtggttagcaaaacaggagactgggtggcaaagtggacctccacctccatgccctgggcagccgccaaggacggcaagctgcactttggaattgatcctgacgatactactatcaccgaccttccctaagccgctggaagattgtattccagatgctagcttagaggtcaagtacagtctcctcatgagacatagcctaatcaattagatctagaattggaaaaattgtcccgtctgtcacttgttttgttgccttaataagcatctgaatgtttggttgtggggcgggttttgaagcgatgagagaaatgcccgtattaggaggattacttgagccctggaggtcaaagctgaggtgagccatgattactccactgcactccagcctgggcaacagagccaggccctgtatcaaaaaaaaaaaaaaaaaaaaaaaaaaaa

SEQ ID NO: 7 - DNA, 1331 bp, Sequência Artificial
  misc_feature (30)..(30): n é t ou c
cggggagcggcggtaccgggcggctgcganctggctcgacccagcttgaggtctcggcgtccgcgtcctgcggtgccctgggatccgccgacatgaatcccatcgtagtggtccacggcggcggagccggtcccatctccaaggatcggaaggagcgagtgcaccagggcatggtcagagccgccaccgtgggctacggcatcctccgggagggcgggagcgccgtggatgccgtagagggagctgtcgtcgccctggaagacgatcccgagttcaacgcaggttgtgggtctgtcttgaacacaaatggtgaggttgaaatggatgctagtatcatggatggaaaagacctgtctgcaggagcagtgtccgcagtccagtgtatagcaaatcccattaaacttgctcggcttgtcatggaaaagacacctcattgctttctgactgaccaaggcgcagcgcagtttgcagcagctatgggggttccagagattcctggagaaaaactggtgacagagagaaacaaaaagcgcctggaaaaagagaagcatgaaaaaggtgctcagaaaacagattgtcaaaaaaacttgggaaccgtgggtgctgttgccttggactgcaaagggaatgtaacctacgcaacctccacaggcggtatcgttaataaaatggtcggccgcgttggggactcaccgtgtctaggagctggaggttatgccgacaatgacatcggagccgtctcaaccacagggcatggggaaagcatcctgaaggtgaacctggctagactcaccctgttccacatagaacaaggaaagacggtagaagaggctgcggacctatcgttgggttatatgaagtcaagggttaaaggtttaggtggcctcatcgtggttagcaaaacaggagactgggtggcaaagtggacctccacctccatgccctgggcagccgccaaggacggcaagctgcactttggaattgatcctgacgatactactatcaccgaccttccctaagccgctggaagattgtattccagatgctagcttagaggtcaagtacagtctcctcatgagacatagcctaatcaattagatctagaattggaaaaattgtcccgtctgtcacttgttttgttgccttaataagcatctgaatgtttggttgtggggcgggttttgaagcgatgagagaaatgcccgtattaggaggattacttgagccctggaggtcaaagctgaggtgagccatgattactccactgcactccagcctgggcaacagagccaggccctgtatcaaaaaaaaaaaaaaaaaaaaaaaaaaaa

SEQ ID NO: 8 - DNA, 1332 bp, Sequência Artificial
  misc_feature (30)..(30): n é t ou c
cggggagcggcggtaccgggcggctgccangctggctcgacccagcttgaggtctcggcgtccgcgtcctgcggtgccctgggatccgccgacatgaatcccatcgtagtggtccacggcggcggagccggtcccatctccaaggatcggaaggagcgagtgcaccagggcatggtcagagccgccaccgtgggctacggcatcctccgggagggcgggagcgccgtggatgccgtagagggagctgtcgtcgccctggaagacgatcccgagttcaacgcaggttgtgggtctgtcttgaacacaaatggtgaggttgaaatggatgctagtatcatggatggaaaagacctgtctgcaggagcagtgtccgcagtccagtgtatagcaaatcccattaaacttgctcggcttgtcatggaaaagacacctcattgctttctgactgaccaaggcgcagcgcagtttgcagcagctatgggggttccagagattcctggagaaaaactggtgacagagagaaacaaaaagcgcctggaaaaagagaagcatgaaaaaggtgctcagaaaacagattgtcaaaaaaacttgggaaccgtgggtgctgttgccttggactgcaaagggaatgtaacctacgcaacctccacaggcggtatcgttaataaaatggtcggccgcgttggggactcaccgtgtctaggagctggaggttatgccgacaatgacatcggagccgtctcaaccacagggcatggggaaagcatcctgaaggtgaacctggctagactcaccctgttccacatagaacaaggaaagacggtagaagaggctgcggacctatcgttgggttatatgaagtcaagggttaaaggtttaggtggcctcatcgtggttagcaaaacaggagactgggtggcaaagtggacctccacctccatgccctgggcagccgccaaggacggcaagctgcactttggaattgatcctgacgatactactatcaccgaccttccctaagccgctggaagattgtattccagatgctagcttagaggtcaagtacagtctcctcatgagacatagcctaatcaattagatctagaattggaaaaattgtcccgtctgtcacttgttttgttgccttaataagcatctgaatgtttggttgtggggcgggttttgaagcgatgagagaaatgcccgtattaggaggattacttgagccctggaggtcaaagctgaggtgagccatgattactccactgcactccagcctgggcaacagagccaggccctgtatcaaaaaaaaaaaaaaaaaaaaaaaaaaaa

SEQ ID NO: 9 - DNA, 24 bp, Sequência Artificial
  Iniciador
catatgaatcccatcgtagtggtc

SEQ ID NO: 10 - DNA, 39 bp, Sequência Artificial
  iniciador
catatgaatcccatcgtagtggtccacggcgaaggagcc

SEQ ID NO: 11 - DNA, 27 bp, Sequência Artificial
  iniciador
ctcgagttagggaaggtcggtgatagt